European Patent Application EP 4 272 764 A1, published November 8, 2023. Title: METHOD OF COMPLEXING BIOLOGICAL UNITS WITH PARTICLES. Applicant: SCIPIO BIOSCIENCE. The sequence listing filed with the application follows.

SEQUENCE LISTING (1 sequence)

SEQ ID NO: 1 - DNA, 34 bp, Artificial Sequence
  dN-Smart Randomer (dN SMRT) oligo
  misc_feature 26: /note="n" is A or G or C or T"
  misc_feature 27: /note="n" is A or G or C or T"
  misc_feature 28: /note="n" is A or G or C or T"
  misc_feature 31: /note="n" is A or G or C or T"
  misc_feature 32: /note="n" is A or G or C or T"
  misc_feature 33: /note="n" is A or G or C or T"
  misc_feature 34: /note="b" is G or C or T"
aagcagtggtatcaacgcagagtgannnggnnnb